European Patent Specification EP 3 881 859 B1, published March 6, 2024. Title: METHODS AND COMPOSITIONS FOR INCREASING NEUROGENESIS AND ANGIOGENESIS. Applicant: President and Fellows of Harvard College The Brigham and Women's Hospital, Inc. Application PCT/US2014/041952. The sequence listing filed with the application follows.

SEQUENCE LISTING (5 sequences)

SEQ ID NO: 1 - protein, 407 aa, Homo sapiens
MVLAAPLLLGFLLLALELRPRGEAAEGPAAAAAAAAAAAAAGVGGERSSRPAPSVAPEPDGCPVCVWRQHSRELRLESIKSQILSKLRLKEAPNISREVVKQLLPKAPPLQQILDLHDFQGDALQPEDFLEEDEYHATTETVISMAQETDPAVQTDGSPLCCHFHFSPKVMFTKVLKAQLWVYLRPVPRPATVYLQILRLKPLTGEGTAGGGGGGRRHIRIRSLKIELHSRSGHWQSIDFKQVLHSWFRQPQSNWGIEINAFDPSGTDLAVTSLGPGAEGLHPFMELRVLENTKRSRRNLGLDCDEHSSESRCCRYPLTVDFEAFGWDWIIAPKRYKANYCSGQCEYMFMQKYPHTHLVQQANPRGSAGPCCTPTKMSPINMLYFNDKQQIIYGKIPGMVVDRCGCS

SEQ ID NO: 2 - protein, 383 aa, Homo sapiens
AEGPAAAAAAAAAAAAAGVGGERSSRPAPSVAPEPDGCPVCVWRQHSRELRLESIKSQILSKLRLKEAPNISREVVKQLLPKAPPLQQILDLHDFQGDALQPEDFLEEDEYHATTETVISMAQETDPAVQTDGSPLCCHFHFSPKVMFTKVLKAQLWVYLRPVPRPATVYLQILRLKPLTGEGTAGGGGGGRRHIRIRSLKIELHSRSGHWQSIDFKQVLHSWFRQPQSNWGIEINAFDPSGTDLAVTSLGPGAEGLHPFMELRVLENTKRSRRNLGLDCDEHSSESRCCRYPLTVDFEAFGWDWIIAPKRYKANYCSGQCEYMFMQKYPHTHLVQQANPRGSAGPCCTPTKMSPINMLYFNDKQQIIYGKIPGMVVDRCGCS

SEQ ID NO: 3 - protein, 109 aa, Homo sapiens
NLGLDCDEHSSESRCCRYPLTVDFEAFGWDWIIAPKRYKANYCSGQCEYMFMQKYPHTHLVQQANPRGSAGPCCTPTKMSPINMLYFNDKQQIIYGKIPGMVVDRCGCS

SEQ ID NO: 4 - protein, 274 aa, Homo sapiens
AEGPAAAAAAAAAAAAAGVGGERSSRPAPSVAPEPDGCPVCVWRQHSRELRLESIKSQILSKLRLKEAPNISREVVKQLLPKAPPLQQILDLHDFQGDALQPEDFLEEDEYHATTETVISMAQETDPAVQTDGSPLCCHFHFSPKVMFTKVLKAQLWVYLRPVPRPATVYLQILRLKPLTGEGTAGGGGGGRRHIRIRSLKIELHSRSGHWQSIDFKQVLHSWFRQPQSNWGIEINAFDPSGTDLAVTSLGPGAEGLHPFMELRVLENTKRSRR

SEQ ID NO: 5 - DNA, 4260 bp, Homo sapiens
tccccgccccccagtcctccctcccctcccctccagcatggtgctcgcggccccgctgctgctgggcttcctgctcctcgccctggagctgcggccccggggggaggcggccgagggccccgcggcggcggcggcggcggcggcggcggcggcagcggcgggggtcgggggggagcgctccagccggccagccccgtccgtggcgcccgagccggacggctgccccgtgtgcgtttggcggcagcacagccgcgagctgcgcctagagagcatcaagtcgcagatcttgagcaaactgcggctcaaggaggcgcccaacatcagccgcgaggtggtgaagcagctgctgcccaaggcgccgccgctgcagcagatcctggacctacacgacttccagggcgacgcgctgcagcccgaggacttcctggaggaggacgagtaccacgccaccaccgagaccgtcattagcatggcccaggagacggacccagcagtacagacagatggcagccctctctgctgccattttcacttcagccccaaggtgatgttcacaaaggtactgaaggcccagctgtgggtgtacctacggcctgtaccccgcccagccacagtctacctgcagatcttgcgactaaaacccctaactggggaagggaccgcagggggagggggcggaggccggcgtcacatccgtatccgctcactgaagattgagctgcactcacgctcaggccattggcagagcatcgacttcaagcaagtgctacacagctggttccgccagccacagagcaactggggcatcgagatcaacgcctttgatcccagtggcacagacctggctgtcacctccctggggccgggagccgaggggctgcatccattcatggagcttcgagtcctagagaacacaaaacgttcccggcggaacctgggtctggactgcgacgagcactcaagcgagtcccgctgctgccgatatcccctcacagtggactttgaggctttcggctgggactggatcatcgcacctaagcgctacaaggccaactactgctccggccagtgcgagtacatgttcatgcaaaaatatccgcatacccatttggtgcagcaggccaatccaagaggctctgctgggccctgttgtacccccaccaagatgtccccaatcaacatgctctacttcaatgacaagcagcagattatctacggcaagatccctggcatggtggtggatcgctgtggctgctcttaaggtgggggatagaggatgcctcccccacagaccctaccccaagacccctagccctgcccccatccccccaagccctagagctccctccactcttcccgcgaacatcacaccgttccccgaccaagccgtgtgcaatacaacagagggaggcaggtgggaattgagggtgaggggtttgggggaaaggggaagcaggggcatagtcagggtggggagtgtttgaagtttgcagatgagaaggtttgacaaaaagacagagagatgtagagacagtgatagagacagaggaacaaaaagagcagcagtgagaaggcaaagagagaggcagaagagacagacgaggcagagacaaaacactgagaaagagactgaaatggagtaataaatgaaagccccacaccaagcctcctttcttccactggcaaggtgaggggcttggtatagtttggggagatcccctgactattcagtaggagaagaaatcaaaaatccattcttttctccttctctccctccaacagtggccaggggaaggggaagtgagggcaggggcaaaaagatttgggaatttttatttatttatttattgtgacttttcatttttttggtatttggctttactggaataggagggcccctgcccactgtgccccgtttatcccttattccccaaaccctgctctccccaacacctactcacttaagcacttgtataaagcctccagggttgggaatgggagtaaagggcaagagggcggacacatgaagtttagtttctaacccatcatcaccctaactcaaccttttctgagccaaatggcttgaattgaagccagttgtcatggaaatagtaagaggttagggtttaagagctggggatgcgggggtgggagagagaaccctcaacatccaggatctatataatgagagctactttaaaccctcaggtccaccctcatgatgctgagttatttagccagagggtgcagcctgcttatgcccaaattccctcagccaagagagagaccaaagagcctctggaatggccctgctcccagcctctatcttcaggtcaattagagagagtatagagaccccagagtcccctgggtctggaaagcgttaggagaggtcaagaaaggagcagtaaggaggctgaaggttacagggcatttgaatccaaatcactgctctgggctagggaatagagccagcagaccaaggtgggaaggattctggaagggggacattttagtctcctaaccccaaagctcagggtggaagaggggagaacaaggaagcagagtgtataattattttttccttttatttttggaatctaacagtacctggcagcagggaggggaaagtacagtggggaaaagcatctgacaaggccagttagaacagaggatgggaaggatggagactcccgggcttggaaggctaggaagcaggcagagactggttgccatttcaagtcactagctaggcccattcattcctcccacaaccctgacccattctcctctggactcactgtgcctcagtttcttcccctcaatggaatgagaaatgacagcacccgccacagccaagagatgaattctgagcacttaccacgggcactttatggacataaaatacctctcgctgtgggacagataaccagggcaccagagtagtggtgaagagatgtgaggcttaagaggagtcacaggcttcagagtacaagttcccctctgcctcccagctggacagtgcctagaagccaaggagttgagaatctcctgatccacaccctatccttacttcaccaccaggcctcttggctccaggcaagagcttagaggatgtcaggagaggtgggggtaagaatcttcagcaaaactgtcactctaagtagagccagcagttacgggtctgataaaaacagtactgaactaaagtaaagcccaagctggtgagcaaaactggatggctcattcttcccaagagcatgactctcccccttggccagttggtggaaggggcaaaggtatgtgaccacccttgagaaggtgatgttggtgagctttaacatcttattcctattcttatagtgagaaagtgaaacaagatctttcagtagaggaatgggcagggctgttaggctcttcagcttgccttcacccatatagcagctatgctaaccccaagcctctctggccctgttcttcatccttccttctgccccaatcctgaaggacaagacacacccggccatcaacaccactcacatttccttggtggaaggaaaggaacagagaagtgaagaacagatacctccctccaaggtcaaatgcctcgtgatcttggcagagtagggattgggcaataagcatcaggtatcttccctctacagattctagagagctggggcattaaatatgggggacacttagaatacagctccttaaataccaccaaataaagacctttgtgtgtgtgtggtgggtggggggggggcaggggtctttctcttatgaacataaatctgtgagctgaagtctcattcccctgttcctccctacccccaaagaggcacagagtgaagggacttggggggcacagctcagcaacccagtgggagttagcaccccctcccaccttatgatgtgtgtggacctggccagtgcccctctgaacatatcattattagtgtaattatcatttattttgtgtatttgtcacattgtgtgcatgacagcctttgttaagggtgtctgaggagtatggagctgacaggggcattggaatgccaggaaagaacttcttcaactgagatcaaggcttcctggagggaaccactgcaaaaaggccatcaggcagttttcaagttatgtgacagagggcaaagacggccatagggtgctctgagttttgggatggtcacatgacacaatccagcacttgaacctgaaaaaaaaaataaaagcggtcaaagagtttagaattca